European Patent Application EP 4 276 174 A1, published November 15, 2023. Title: GENE THERAPY FOR THE TREATMENT OF ACTIVATED PI3KINASE DELTA SYNDROME TYPE 1 (APDS1). Applicant: Cellectis S.A. INSERM (Institut National de la Santé et de la Recherche Médicale) Assistance Publique - Hôpitaux de Paris (APHP) Université Paris Cité Fondation Imagine. The sequence listing filed with the application follows.

SEQUENCE LISTING (46 sequences)

SEQ ID NO: 1 - DNA, 2115 bp, artificial
  Optimized coding sequence Exons8-24
ctggtggtgcaggcaggactgttccacggaaacgagatgctgtgcaagaccgtgagctcctctgaggtgagcgtgtgctctgagcccgtgtggaagcagaggctggagttcgacatcaatatctgcgatctgccacggatggccagactgtgctttgccctgtacgccgtgatcgagaaggccaagaaggcccgctccaccaagaagaagagcaagaaggcagactgcccaatcgcatgggcaaacctgatgctgtttgactacaaggatcagctgaagacaggcgagaggtgtctgtatatgtggcctagcgtgccagacgagaagggcgagctgctgaatcccaccggcacagtgcgctctaaccctaataccgatagcgccgccgccctgctgatctgcctgccagaggtggcaccacaccccgtgtactatcccgccctggagaagatcctggagctgggcaggcacagcgagtgcgtgcacgtgacagaggaggagcagctgcagctgagggagatcctggagaggagaggatccggcgagctgtacgagcacgagaaggacctggtgtggaagctgcggcacgaggtgcaggagcacttcccagaggccctggcaagactgctgctggtgaccaagtggaacaagcacgaggatgtggcccagatgctgtatctgctgtgcagctggccagagctgcctgtgctgtccgccctggagctgctggacttctcttttcctgattgtcacgtgggcagcttcgccatcaagtccctgcggaagctgaccgacgatgagctgtttcagtacctgctgcagctggtgcaggtgctgaagtacgagagctatctggactgcgagctgacaaagttcctgctggatagggccctggccaaccgcaagatcggccacttcctgttttggcacctgagatccgagatgcacgtgccttctgtggccctgaggtttggcctgatcctggaggcctattgtcgcggctctacccaccacatgaaggtgctgatgaagcagggcgaggccctgagcaagctgaaggccctgaatgactttgtgaagctgagctcccagaagaccccaaagccccagacaaaggagctgatgcacctgtgcatgaggcaggaggcctacctggaggccctgtctcacctgcagagcccactggacccatccaccctgctggcagaggtgtgcgtggagcagtgtacattcatggattctaagatgaagccactgtggatcatgtatagcaacgaggaggcaggaagcggaggatccgtgggcatcatctttaagaatggcgacgatctgcggcaggatatgctgaccctgcagatgatccagctgatggacgtgctgtggaagcaggagggcctggatctgagaatgacaccttacggatgcctgccaaccggcgacaggacaggactgatcgaggtggtgctgagatccgataccatcgccaacatccagctgaacaagtctaatatggccgccacagccgccttcaataaggacgccctgctgaactggctgaagtccaagaatcctggagaggccctggatagggcaatcgaggagtttaccctgtcttgcgccggctactgcgtggccacatatgtgctgggcatcggcgaccggcacagcgataatatcatgatcagagagtccggccagctgttccacatcgacttcggccactttctgggcaacttcaagaccaagtttggcatcaatcgggagagagtgccattcatcctgacctacgattttgtgcacgtgatccagcagggcaagacaaacaattctgagaagttcgagaggtttcgcggctactgcgagcgggcctatacaatcctgaggcgccacggcctgctgttcctgcacctgtttgcactgatgagagcagcaggactgccagagctgtcttgtagcaaggacatccagtatctgaaggattccctggccctgggcaagaccgaggaggaggccctgaagcacttcagggtgaagtttaacgaggccctgcgcgagagctggaagacaaaggtgaactggctggcccacaacgtgagcaaggacaaccggcagtaa

SEQ ID NO: 2 - DNA, 972 bp, artificial
  Optimized coding sequence Exons17-24
gaggcctacctggaggccctgtcccacctgcagtctccactggaccctagcaccctgctggcagaggtgtgcgtggagcagtgtacattcatggattctaagatgaagcccctgtggatcatgtatagcaacgaggaggcaggatctggaggaagcgtgggcatcatctttaagaatggcgacgatctgaggcaggacatgctgaccctgcagatgatccagctgatggacgtgctgtggaagcaggagggcctggatctgcgcatgacaccatacggatgcctgccaaccggcgacaggacaggcctgatcgaggtggtgctgcgctccgataccatcgccaacatccagctgaacaagtctaatatggccgccacagccgccttcaataaggacgccctgctgaactggctgaagtctaagaatcctggagaggccctggatagggcaatcgaggagtttaccctgagctgcgcaggatactgcgtggcaacatatgtgctgggcatcggcgacaggcacagcgataatatcatgatccgcgagtccggccagctgttccacatcgacttcggccactttctgggcaacttcaagaccaagtttggcatcaatagggagcgcgtgcctttcatcctgacctacgattttgtgcacgtgatccagcagggcaagacaaacaattccgagaagttcgagcggtttagaggctactgcgagcgggcctataccatcctgcggagacacggcctgctgttcctgcacctgtttgcactgatgagagcagcaggactgccagagctgagctgttccaaggacatccagtatctgaaggattctctggccctgggcaagaccgaggaggaggccctgaagcacttccgggtgaagtttaacgaggccctgagagagagctggaagacaaaggtgaactggctggcccacaacgtgagcaaggataacaggcagtaa

SEQ ID NO: 3 - DNA, 47 bp, artificial
  Exon8 TALEN target
tgaacgccgacgagcggatgaaggtggggctcctgggataggtggga

SEQ ID NO: 4 - DNA, 17 bp, artificial
  Exon8 TALEN target Left
tgaacgccgacgagcgg

SEQ ID NO: 5 - DNA, 17 bp, artificial
  Exon8 TALEN target Right
tcccacctatcccagga

SEQ ID NO: 6 - DNA, 49 bp, artificial
  Exon17 TALEN target
tgatgcacttgtgcatgcggcaggaggcctacctagaggccctctccca

SEQ ID NO: 7 - DNA, 17 bp, artificial
  Exon17 TALEN target Left
tgatgcacttgtgcatg

SEQ ID NO: 8 - DNA, 17 bp, artificial
  Exon17 TALEN target Right
tgggagagggcctctag

SEQ ID NO: 9 - DNA, 57 bp, artificial
  Exon24 TALEN target
tggcactggggaaaacagaggaggaggcactgaagcacttccgagtgaagtttaaca

SEQ ID NO: 10 - DNA, 17 bp, artificial
  Exon24 TALEN target Left
tggcactggggaaaaca

SEQ ID NO: 11 - DNA, 17 bp, artificial
  Exon24 TALEN target Right
tgttaaacttcactcgg

SEQ ID NO: 12 - DNA, 300 bp, artificial
  left homology for Exon8 donor template
cccctctgcagagctcaggggtgttggggccccctggggagcccgcatggcaggttttctgggaaaggatagcattgtggacaggcccaaacctggccgcaaacctgtgaccctctcacccgcccccaagtggtcacgggcctcaccataggccagggagacaagctgcactttgagccgtgttaacagccctgcttccccggcccccagccttcctctgtgtccctgtggtccctggagcagccgttccgcatcgagctcatccagggcagcaaagtgaacgccgacgagcggatgaag

SEQ ID NO: 13 - DNA, 300 bp, artificial
  right homology for Exon8 donor template
gtggggctcctgggataggtgggagagacactgtttttttgcacaaacaaggtggctgtatcctggaggggtagcagaggaaggagggggatcacatgaaagccacctgaccacattacccagcatccctgcctggggcgctgtgagcggcttgaaaacaggaagtggggagggggtgggccagccggccctggaggctgattcgtagaaacttgggccaagcagcgttctgggtatttgactttggtggaggttatggggccaggttcagcccagggatccgggaccgcagagctgggg

SEQ ID NO: 14 - DNA, 500 bp, artificial
  left homology for Exon17 donor template
ctccggtagcgggacttgccccagccgttctgtgggaatcccagcccctgagtctccctggaaggccactggggacgtttccagcaggcctgggtgtcctggcctcgctaggtcctgctgggcgggaggggctgcgtggtgctgcctggtgaggctcagccctcccttcaccttccagctccgagatgcacgtgccgtcggtggccctgcgcttcggcctcatcctggaggcctactgcaggggcagcacccaccacatgaaggtgctgatgaagcaggtgaggcccaaggccctggggggcgggcagggggcggccctgagcgtctgggaatccccagggctgggtcgaggctgggacctgcccaccgccgccctcccatctgcccaccagggggaagcactgagcaaactgaaggccctgaatgacttcgtcaagctgagctctcagaagacccccaagccccagaccaaggagctgatgcacttgtgcatgcggcag

SEQ ID NO: 15 - DNA, 500 bp, artificial
  right homology for Exon17 donor template
gaggcctacctagaggccctctcccacctgcagtccccactcgaccccagcaccctgctggctgaagtctggtgagcccaagccccgccacaagggttcctcccacccctgggaggccggtagaggagcccctgctgactgcccgctctctggcctggcagcgtggagcagtgcaccttcatggactccaagatgaagcccctgtggatcatgtacagcaacgaggaggcaggcagcggcggcagcgtgggcatcatctttaagaacggggatggtgagggcctggcctccccacaccccgcctgtactgccctggggggtcctggggtgctcctagagtgggggtggagaagacagaatcctgggacttaagggcttgggtgtagctggaagcagagaacctaccagaaactcacgcttctcctcccaccggccggtggcacagacctccggcaggacatgctgaccctgcagatgatccagctcatggacgtcctgtg

SEQ ID NO: 16 - DNA, 228 bp, artificial
  BGH polyA
cgactgtgccttctagttgccagccatctgttgtttgcccctcccccgtgccttccttgaccctggaaggtgccactcccactgtcctttcctaataaaatgaggaaattgcatcgcattgtctgagtaggtgtcattctattctggggggtggggtggggcaggacagcaagggggaggattgggaagacaatagcaggcatgctggggatgcggtgggctctatgg

SEQ ID NO: 17 - DNA, 246 bp, artificial
  SV40 polyA
gcagatccagacatgataagatacattgatgagtttggacaaaccacaactagaatgcagtgaaaaaaatgctttatttgtgaaatttgtgatgctattgctttatttgtaaccattataagctgcaataaacaagttaacaacaacaattgcattcattttatgtttcaggttcagggggaggtgtgggaggttttttaaagcaagtaaaacctctacaaatgtggtacggcttgattatgatca

SEQ ID NO: 18 - DNA, 253 bp, artificial
  EF1a promoter
ggatctgcgatcgctccggtgcccgtcagtgggcagagcgcacatcgcccacagtccccgagaagttggggggaggggtcggcaattgaaccggtgcctagagaaggtggcgcggggtaaactgggaaagtgatgtcgtgtactggctccgcctttttcccgagggtgggggagaaccgtatataagtgcagtagtcgccgtgaacgttctttttcgcaacgggtttgccgccagaacacagtcgacgccacc

SEQ ID NO: 19 - DNA, 545 bp, artificial
  PGK promoter
ggggttggggttgcgccttttccaaggcagccctgggtttgcgcagggacgcggctgctctgggcgtggttccgggaaacgcagcggcgccgaccctgggtctcgcacattcttcacgtccgttcgcagcgtcacccggatcttcgccgctacccttgtgggccccccggcgacgcttcctgctccgcccctaagtcgggaaggttccttgcggttcgcggcgtgccggacgtgacaaacggaagccgcacgtctcactagtaccctcgcagacggacagcgccagggagcaatggcagcgcgccgaccgcgatgggctgtggccaatagcggctgctcagcagggcgcgccgagagcagcggccgggaaggggcggtgcgggaggcggggtgtggggcggtagtgtgggccctgttcctgcccgcgcggtgttccgcattctgcaagcctccggagcgcacgtcggcagtcggctccctcgttgaccgaatcaccgacctctctccccagggggatccaccggtcgccaccggtcgacgccacc

SEQ ID NO: 20 - DNA, 66 bp, artificial
  P2A
ggaagcggagctactaacttcagcctgctgaagcaggctggagacgtggaggagaaccctggacct

SEQ ID NO: 21 - DNA, 825 bp, artificial
  truncated LNGFR reporter gene
atgggggcaggtgccaccggccgcgccatggacgggccgcgcctgctgctgttgctgcttctgggggtgtcccttggaggtgccaaggaggcatgccccacaggcctgtacacacacagcggtgagtgctgcaaagcctgcaacctgggcgagggtgtggcccagccttgtggagccaaccagaccgtgtgtgagccctgcctggacagcgtgacgttctccgacgtggtgagcgcgaccgagccgtgcaagccgtgcaccgagtgcgtggggctccagagcatgtcggcgccgtgcgtggaggccgatgacgccgtgtgccgctgcgcctacggctactaccaggatgagacgactgggcgctgcgaggcgtgccgcgtgtgcgaggcgggctcgggcctcgtgttctcctgccaggacaagcagaacaccgtgtgcgaggagtgccccgacggcacgtattccgacgaggccaaccacgtggacccgtgcctgccctgcaccgtgtgcgaggacaccgagcgccagctccgcgagtgcacacgctgggccgacgccgagtgcgaggagatccctggccgttggattacacggtccacacccccagagggctcggacagcacagcccccagcacccaggagcctgaggcacctccagaacaagacctcatagccagcacggtggcaggtgtggtgaccacagtgatgggcagctcccagcccgtggtgacccgaggcaccaccgacaacctcatccctgtctattgctccatcctggctgctgtggttgtgggtcttgtggcctacatagccttcaagaggtga

SEQ ID NO: 22 - DNA, 4267 bp, artificial
  Exon8 donor template EF1a
cccctctgcagagctcaggggtgttggggccccctggggagcccgcatggcaggttttctgggaaaggatagcattgtggacaggcccaaacctggccgcaaacctgtgaccctctcacccgcccccaagtggtcacgggcctcaccataggccagggagacaagctgcactttgagccgtgttaacagccctgcttccccggcccccagccttcctctgtgtccctgtggtccctggagcagccgttccgcatcgagctcatccagggcagcaaagtgaacgccgacgagcggatgaagctggtggtgcaggcaggactgttccacggaaacgagatgctgtgcaagaccgtgagctcctctgaggtgagcgtgtgctctgagcccgtgtggaagcagaggctggagttcgacatcaatatctgcgatctgccacggatggccagactgtgctttgccctgtacgccgtgatcgagaaggccaagaaggcccgctccaccaagaagaagagcaagaaggcagactgcccaatcgcatgggcaaacctgatgctgtttgactacaaggatcagctgaagacaggcgagaggtgtctgtatatgtggcctagcgtgccagacgagaagggcgagctgctgaatcccaccggcacagtgcgctctaaccctaataccgatagcgccgccgccctgctgatctgcctgccagaggtggcaccacaccccgtgtactatcccgccctggagaagatcctggagctgggcaggcacagcgagtgcgtgcacgtgacagaggaggagcagctgcagctgagggagatcctggagaggagaggatccggcgagctgtacgagcacgagaaggacctggtgtggaagctgcggcacgaggtgcaggagcacttcccagaggccctggcaagactgctgctggtgaccaagtggaacaagcacgaggatgtggcccagatgctgtatctgctgtgcagctggccagagctgcctgtgctgtccgccctggagctgctggacttctcttttcctgattgtcacgtgggcagcttcgccatcaagtccctgcggaagctgaccgacgatgagctgtttcagtacctgctgcagctggtgcaggtgctgaagtacgagagctatctggactgcgagctgacaaagttcctgctggatagggccctggccaaccgcaagatcggccacttcctgttttggcacctgagatccgagatgcacgtgccttctgtggccctgaggtttggcctgatcctggaggcctattgtcgcggctctacccaccacatgaaggtgctgatgaagcagggcgaggccctgagcaagctgaaggccctgaatgactttgtgaagctgagctcccagaagaccccaaagccccagacaaaggagctgatgcacctgtgcatgaggcaggaggcctacctggaggccctgtctcacctgcagagcccactggacccatccaccctgctggcagaggtgtgcgtggagcagtgtacattcatggattctaagatgaagccactgtggatcatgtatagcaacgaggaggcaggaagcggaggatccgtgggcatcatctttaagaatggcgacgatctgcggcaggatatgctgaccctgcagatgatccagctgatggacgtgctgtggaagcaggagggcctggatctgagaatgacaccttacggatgcctgccaaccggcgacaggacaggactgatcgaggtggtgctgagatccgataccatcgccaacatccagctgaacaagtctaatatggccgccacagccgccttcaataaggacgccctgctgaactggctgaagtccaagaatcctggagaggccctggatagggcaatcgaggagtttaccctgtcttgcgccggctactgcgtggccacatatgtgctgggcatcggcgaccggcacagcgataatatcatgatcagagagtccggccagctgttccacatcgacttcggccactttctgggcaacttcaagaccaagtttggcatcaatcgggagagagtgccattcatcctgacctacgattttgtgcacgtgatccagcagggcaagacaaacaattctgagaagttcgagaggtttcgcggctactgcgagcgggcctatacaatcctgaggcgccacggcctgctgttcctgcacctgtttgcactgatgagagcagcaggactgccagagctgtcttgtagcaaggacatccagtatctgaaggattccctggccctgggcaagaccgaggaggaggccctgaagcacttcagggtgaagtttaacgaggccctgcgcgagagctggaagacaaaggtgaactggctggcccacaacgtgagcaaggacaaccggcagtaacgactgtgccttctagttgccagccatctgttgtttgcccctcccccgtgccttccttgaccctggaaggtgccactcccactgtcctttcctaataaaatgaggaaattgcatcgcattgtctgagtaggtgtcattctattctggggggtggggtggggcaggacagcaagggggaggattgggaagacaatagcaggcatgctggggatgcggtgggctctatggggatctgcgatcgctccggtgcccgtcagtgggcagagcgcacatcgcccacagtccccgagaagttggggggaggggtcggcaattgaaccggtgcctagagaaggtggcgcggggtaaactgggaaagtgatgtcgtgtactggctccgcctttttcccgagggtgggggagaaccgtatataagtgcagtagtcgccgtgaacgttctttttcgcaacgggtttgccgccagaacacagtcgacgccaccatgggggcaggtgccaccggccgcgccatggacgggccgcgcctgctgctgttgctgcttctgggggtgtcccttggaggtgccaaggaggcatgccccacaggcctgtacacacacagcggtgagtgctgcaaagcctgcaacctgggcgagggtgtggcccagccttgtggagccaaccagaccgtgtgtgagccctgcctggacagcgtgacgttctccgacgtggtgagcgcgaccgagccgtgcaagccgtgcaccgagtgcgtggggctccagagcatgtcggcgccgtgcgtggaggccgatgacgccgtgtgccgctgcgcctacggctactaccaggatgagacgactgggcgctgcgaggcgtgccgcgtgtgcgaggcgggctcgggcctcgtgttctcctgccaggacaagcagaacaccgtgtgcgaggagtgccccgacggcacgtattccgacgaggccaaccacgtggacccgtgcctgccctgcaccgtgtgcgaggacaccgagcgccagctccgcgagtgcacacgctgggccgacgccgagtgcgaggagatccctggccgttggattacacggtccacacccccagagggctcggacagcacagcccccagcacccaggagcctgaggcacctccagaacaagacctcatagccagcacggtggcaggtgtggtgaccacagtgatgggcagctcccagcccgtggtgacccgaggcaccaccgacaacctcatccctgtctattgctccatcctggctgctgtggttgtgggtcttgtggcctacatagccttcaagaggtgagcagatccagacatgataagatacattgatgagtttggacaaaccacaactagaatgcagtgaaaaaaatgctttatttgtgaaatttgtgatgctattgctttatttgtaaccattataagctgcaataaacaagttaacaacaacaattgcattcattttatgtttcaggttcagggggaggtgtgggaggttttttaaagcaagtaaaacctctacaaatgtggtacggcttgattatgatcagtggggctcctgggataggtgggagagacactgtttttttgcacaaacaaggtggctgtatcctggaggggtagcagaggaaggagggggatcacatgaaagccacctgaccacattacccagcatccctgcctggggcgctgtgagcggcttgaaaacaggaagtggggagggggtgggccagccggccctggaggctgattcgtagaaacttgggccaagcagcgttctgggtatttgactttggtggaggttatggggccaggttcagcccagggatccgggaccgcagagctgggg

SEQ ID NO: 23 - DNA, 3849 bp, artificial
  Exon8 donor template P2A
cccctctgcagagctcaggggtgttggggccccctggggagcccgcatggcaggttttctgggaaaggatagcattgtggacaggcccaaacctggccgcaaacctgtgaccctctcacccgcccccaagtggtcacgggcctcaccataggccagggagacaagctgcactttgagccgtgttaacagccctgcttccccggcccccagccttcctctgtgtccctgtggtccctggagcagccgttccgcatcgagctcatccagggcagcaaagtgaacgccgacgagcggatgaagctggtggtgcaggcaggactgttccacggaaacgagatgctgtgcaagaccgtgagctcctctgaggtgagcgtgtgctctgagcccgtgtggaagcagaggctggagttcgacatcaatatctgcgatctgccacggatggccagactgtgctttgccctgtacgccgtgatcgagaaggccaagaaggcccgctccaccaagaagaagagcaagaaggcagactgcccaatcgcatgggcaaacctgatgctgtttgactacaaggatcagctgaagacaggcgagaggtgtctgtatatgtggcctagcgtgccagacgagaagggcgagctgctgaatcccaccggcacagtgcgctctaaccctaataccgatagcgccgccgccctgctgatctgcctgccagaggtggcaccacaccccgtgtactatcccgccctggagaagatcctggagctgggcaggcacagcgagtgcgtgcacgtgacagaggaggagcagctgcagctgagggagatcctggagaggagaggatccggcgagctgtacgagcacgagaaggacctggtgtggaagctgcggcacgaggtgcaggagcacttcccagaggccctggcaagactgctgctggtgaccaagtggaacaagcacgaggatgtggcccagatgctgtatctgctgtgcagctggccagagctgcctgtgctgtccgccctggagctgctggacttctcttttcctgattgtcacgtgggcagcttcgccatcaagtccctgcggaagctgaccgacgatgagctgtttcagtacctgctgcagctggtgcaggtgctgaagtacgagagctatctggactgcgagctgacaaagttcctgctggatagggccctggccaaccgcaagatcggccacttcctgttttggcacctgagatccgagatgcacgtgccttctgtggccctgaggtttggcctgatcctggaggcctattgtcgcggctctacccaccacatgaaggtgctgatgaagcagggcgaggccctgagcaagctgaaggccctgaatgactttgtgaagctgagctcccagaagaccccaaagccccagacaaaggagctgatgcacctgtgcatgaggcaggaggcctacctggaggccctgtctcacctgcagagcccactggacccatccaccctgctggcagaggtgtgcgtggagcagtgtacattcatggattctaagatgaagccactgtggatcatgtatagcaacgaggaggcaggaagcggaggatccgtgggcatcatctttaagaatggcgacgatctgcggcaggatatgctgaccctgcagatgatccagctgatggacgtgctgtggaagcaggagggcctggatctgagaatgacaccttacggatgcctgccaaccggcgacaggacaggactgatcgaggtggtgctgagatccgataccatcgccaacatccagctgaacaagtctaatatggccgccacagccgccttcaataaggacgccctgctgaactggctgaagtccaagaatcctggagaggccctggatagggcaatcgaggagtttaccctgtcttgcgccggctactgcgtggccacatatgtgctgggcatcggcgaccggcacagcgataatatcatgatcagagagtccggccagctgttccacatcgacttcggccactttctgggcaacttcaagaccaagtttggcatcaatcgggagagagtgccattcatcctgacctacgattttgtgcacgtgatccagcagggcaagacaaacaattctgagaagttcgagaggtttcgcggctactgcgagcgggcctatacaatcctgaggcgccacggcctgctgttcctgcacctgtttgcactgatgagagcagcaggactgccagagctgtcttgtagcaaggacatccagtatctgaaggattccctggccctgggcaagaccgaggaggaggccctgaagcacttcagggtgaagtttaacgaggccctgcgcgagagctggaagacaaaggtgaactggctggcccacaacgtgagcaaggacaaccggcagggaagcggagctactaacttcagcctgctgaagcaggctggagacgtggaggagaaccctggacctatgggggcaggtgccaccggccgcgccatggacgggccgcgcctgctgctgttgctgcttctgggggtgtcccttggaggtgccaaggaggcatgccccacaggcctgtacacacacagcggtgagtgctgcaaagcctgcaacctgggcgagggtgtggcccagccttgtggagccaaccagaccgtgtgtgagccctgcctggacagcgtgacgttctccgacgtggtgagcgcgaccgagccgtgcaagccgtgcaccgagtgcgtggggctccagagcatgtcggcgccgtgcgtggaggccgatgacgccgtgtgccgctgcgcctacggctactaccaggatgagacgactgggcgctgcgaggcgtgccgcgtgtgcgaggcgggctcgggcctcgtgttctcctgccaggacaagcagaacaccgtgtgcgaggagtgccccgacggcacgtattccgacgaggccaaccacgtggacccgtgcctgccctgcaccgtgtgcgaggacaccgagcgccagctccgcgagtgcacacgctgggccgacgccgagtgcgaggagatccctggccgttggattacacggtccacacccccagagggctcggacagcacagcccccagcacccaggagcctgaggcacctccagaacaagacctcatagccagcacggtggcaggtgtggtgaccacagtgatgggcagctcccagcccgtggtgacccgaggcaccaccgacaacctcatccctgtctattgctccatcctggctgctgtggttgtgggtcttgtggcctacatagccttcaagaggtgagcagatccagacatgataagatacattgatgagtttggacaaaccacaactagaatgcagtgaaaaaaatgctttatttgtgaaatttgtgatgctattgctttatttgtaaccattataagctgcaataaacaagttaacaacaacaattgcattcattttatgtttcaggttcagggggaggtgtgggaggttttttaaagcaagtaaaacctctacaaatgtggtacggcttgattatgatcagtggggctcctgggataggtgggagagacactgtttttttgcacaaacaaggtggctgtatcctggaggggtagcagaggaaggagggggatcacatgaaagccacctgaccacattacccagcatccctgcctggggcgctgtgagcggcttgaaaacaggaagtggggagggggtgggccagccggccctggaggctgattcgtagaaacttgggccaagcagcgttctgggtatttgactttggtggaggttatggggccaggttcagcccagggatccgggaccgcagagctgggg

SEQ ID NO: 24 - DNA, 3816 bp, artificial
  Exon17 donor template EF1a
ctccggtagcgggacttgccccagccgttctgtgggaatcccagcccctgagtctccctggaaggccactggggacgtttccagcaggcctgggtgtcctggcctcgctaggtcctgctgggcgggaggggctgcgtggtgctgcctggtgaggctcagccctcccttcaccttccagctccgagatgcacgtgccgtcggtggccctgcgcttcggcctcatcctggaggcctactgcaggggcagcacccaccacatgaaggtgctgatgaagcaggtgaggcccaaggccctggggggcgggcagggggcggccctgagcgtctgggaatccccagggctgggtcgaggctgggacctgcccaccgccgccctcccatctgcccaccagggggaagcactgagcaaactgaaggccctgaatgacttcgtcaagctgagctctcagaagacccccaagccccagaccaaggagctgatgcacttgtgcatgcggcaggaggcctacctggaggccctgtcccacctgcagtctccactggaccctagcaccctgctggcagaggtgtgcgtggagcagtgtacattcatggattctaagatgaagcccctgtggatcatgtatagcaacgaggaggcaggatctggaggaagcgtgggcatcatctttaagaatggcgacgatctgaggcaggacatgctgaccctgcagatgatccagctgatggacgtgctgtggaagcaggagggcctggatctgcgcatgacaccatacggatgcctgccaaccggcgacaggacaggcctgatcgaggtggtgctgcgctccgataccatcgccaacatccagctgaacaagtctaatatggccgccacagccgccttcaataaggacgccctgctgaactggctgaagtctaagaatcctggagaggccctggatagggcaatcgaggagtttaccctgagctgcgcaggatactgcgtggcaacatatgtgctgggcatcggcgacaggcacagcgataatatcatgatccgcgagtccggccagctgttccacatcgacttcggccactttctgggcaacttcaagaccaagtttggcatcaatagggagcgcgtgcctttcatcctgacctacgattttgtgcacgtgatccagcagggcaagacaaacaattccgagaagttcgagcggtttagaggctactgcgagcgggcctataccatcctgcggagacacggcctgctgttcctgcacctgtttgcactgatgagagcagcaggactgccagagctgagctgttccaaggacatccagtatctgaaggattctctggccctgggcaagaccgaggaggaggccctgaagcacttccgggtgaagtttaacgaggccctgagagagagctggaagacaaaggtgaactggctggcccacaacgtgagcaaggataacaggcagtaacgactgtgccttctagttgccagccatctgttgtttgcccctcccccgtgccttccttgaccctggaaggtgccactcccactgtcctttcctaataaaatgaggaaattgcatcgcattgtctgagtaggtgtcattctattctggggggtggggtggggcaggacagcaagggggaggattgggaagacaatagcaggcatgctggggatgcggtgggctctatggggggttggggttgcgccttttccaaggcagccctgggtttgcgcagggacgcggctgctctgggcgtggttccgggaaacgcagcggcgccgaccctgggtctcgcacattcttcacgtccgttcgcagcgtcacccggatcttcgccgctacccttgtgggccccccggcgacgcttcctgctccgcccctaagtcgggaaggttccttgcggttcgcggcgtgccggacgtgacaaacggaagccgcacgtctcactagtaccctcgcagacggacagcgccagggagcaatggcagcgcgccgaccgcgatgggctgtggccaatagcggctgctcagcagggcgcgccgagagcagcggccgggaaggggcggtgcgggaggcggggtgtggggcggtagtgtgggccctgttcctgcccgcgcggtgttccgcattctgcaagcctccggagcgcacgtcggcagtcggctccctcgttgaccgaatcaccgacctctctccccagggggatccaccggtcgccaccggtcgacgccaccatgggggcaggtgccaccggccgcgccatggacgggccgcgcctgctgctgttgctgcttctgggggtgtcccttggaggtgccaaggaggcatgccccacaggcctgtacacacacagcggtgagtgctgcaaagcctgcaacctgggcgagggtgtggcccagccttgtggagccaaccagaccgtgtgtgagccctgcctggacagcgtgacgttctccgacgtggtgagcgcgaccgagccgtgcaagccgtgcaccgagtgcgtggggctccagagcatgtcggcgccgtgcgtggaggccgatgacgccgtgtgccgctgcgcctacggctactaccaggatgagacgactgggcgctgcgaggcgtgccgcgtgtgcgaggcgggctcgggcctcgtgttctcctgccaggacaagcagaacaccgtgtgcgaggagtgccccgacggcacgtattccgacgaggccaaccacgtggacccgtgcctgccctgcaccgtgtgcgaggacaccgagcgccagctccgcgagtgcacacgctgggccgacgccgagtgcgaggagatccctggccgttggattacacggtccacacccccagagggctcggacagcacagcccccagcacccaggagcctgaggcacctccagaacaagacctcatagccagcacggtggcaggtgtggtgaccacagtgatgggcagctcccagcccgtggtgacccgaggcaccaccgacaacctcatccctgtctattgctccatcctggctgctgtggttgtgggtcttgtggcctacatagccttcaagaggtgagcagatccagacatgataagatacattgatgagtttggacaaaccacaactagaatgcagtgaaaaaaatgctttatttgtgaaatttgtgatgctattgctttatttgtaaccattataagctgcaataaacaagttaacaacaacaattgcattcattttatgtttcaggttcagggggaggtgtgggaggttttttaaagcaagtaaaacctctacaaatgtggtacggcttgattatgatcagaggcctacctagaggccctctcccacctgcagtccccactcgaccccagcaccctgctggctgaagtctggtgagcccaagccccgccacaagggttcctcccacccctgggaggccggtagaggagcccctgctgactgcccgctctctggcctggcagcgtggagcagtgcaccttcatggactccaagatgaagcccctgtggatcatgtacagcaacgaggaggcaggcagcggcggcagcgtgggcatcatctttaagaacggggatggtgagggcctggcctccccacaccccgcctgtactgccctggggggtcctggggtgctcctagagtgggggtggagaagacagaatcctgggacttaagggcttgggtgtagctggaagcagagaacctaccagaaactcacgcttctcctcccaccggccggtggcacagacctccggcaggacatgctgaccctgcagatgatccagctcatggacgtcctgtg

SEQ ID NO: 25 - DNA, 3106 bp, artificial
  Exon17 donor template P2A
ctccggtagcgggacttgccccagccgttctgtgggaatcccagcccctgagtctccctggaaggccactggggacgtttccagcaggcctgggtgtcctggcctcgctaggtcctgctgggcgggaggggctgcgtggtgctgcctggtgaggctcagccctcccttcaccttccagctccgagatgcacgtgccgtcggtggccctgcgcttcggcctcatcctggaggcctactgcaggggcagcacccaccacatgaaggtgctgatgaagcaggtgaggcccaaggccctggggggcgggcagggggcggccctgagcgtctgggaatccccagggctgggtcgaggctgggacctgcccaccgccgccctcccatctgcccaccagggggaagcactgagcaaactgaaggccctgaatgacttcgtcaagctgagctctcagaagacccccaagccccagaccaaggagctgatgcacttgtgcatgcggcaggaggcctacctggaggccctgtcccacctgcagtctccactggaccctagcaccctgctggcagaggtgtgcgtggagcagtgtacattcatggattctaagatgaagcccctgtggatcatgtatagcaacgaggaggcaggatctggaggaagcgtgggcatcatctttaagaatggcgacgatctgaggcaggacatgctgaccctgcagatgatccagctgatggacgtgctgtggaagcaggagggcctggatctgcgcatgacaccatacggatgcctgccaaccggcgacaggacaggcctgatcgaggtggtgctgcgctccgataccatcgccaacatccagctgaacaagtctaatatggccgccacagccgccttcaataaggacgccctgctgaactggctgaagtctaagaatcctggagaggccctggatagggcaatcgaggagtttaccctgagctgcgcaggatactgcgtggcaacatatgtgctgggcatcggcgacaggcacagcgataatatcatgatccgcgagtccggccagctgttccacatcgacttcggccactttctgggcaacttcaagaccaagtttggcatcaatagggagcgcgtgcctttcatcctgacctacgattttgtgcacgtgatccagcagggcaagacaaacaattccgagaagttcgagcggtttagaggctactgcgagcgggcctataccatcctgcggagacacggcctgctgttcctgcacctgtttgcactgatgagagcagcaggactgccagagctgagctgttccaaggacatccagtatctgaaggattctctggccctgggcaagaccgaggaggaggccctgaagcacttccgggtgaagtttaacgaggccctgagagagagctggaagacaaaggtgaactggctggcccacaacgtgagcaaggataacaggcagggaagcggagctactaacttcagcctgctgaagcaggctggagacgtggaggagaaccctggacctatgggggcaggtgccaccggccgcgccatggacgggccgcgcctgctgctgttgctgcttctgggggtgtcccttggaggtgccaaggaggcatgccccacaggcctgtacacacacagcggtgagtgctgcaaagcctgcaacctgggcgagggtgtggcccagccttgtggagccaaccagaccgtgtgtgagccctgcctggacagcgtgacgttctccgacgtggtgagcgcgaccgagccgtgcaagccgtgcaccgagtgcgtggggctccagagcatgtcggcgccgtgcgtggaggccgatgacgccgtgtgccgctgcgcctacggctactaccaggatgagacgactgggcgctgcgaggcgtgccgcgtgtgcgaggcgggctcgggcctcgtgttctcctgccaggacaagcagaacaccgtgtgcgaggagtgccccgacggcacgtattccgacgaggccaaccacgtggacccgtgcctgccctgcaccgtgtgcgaggacaccgagcgccagctccgcgagtgcacacgctgggccgacgccgagtgcgaggagatccctggccgttggattacacggtccacacccccagagggctcggacagcacagcccccagcacccaggagcctgaggcacctccagaacaagacctcatagccagcacggtggcaggtgtggtgaccacagtgatgggcagctcccagcccgtggtgacccgaggcaccaccgacaacctcatccctgtctattgctccatcctggctgctgtggttgtgggtcttgtggcctacatagccttcaagaggtgagcagatccagacatgataagatacattgatgagtttggacaaaccacaactagaatgcagtgaaaaaaatgctttatttgtgaaatttgtgatgctattgctttatttgtaaccattataagctgcaataaacaagttaacaacaacaattgcattcattttatgtttcaggttcagggggaggtgtgggaggttttttaaagcaagtaaaacctctacaaatgtggtacggcttgattatgatcagaggcctacctagaggccctctcccacctgcagtccccactcgaccccagcaccctgctggctgaagtctggtgagcccaagccccgccacaagggttcctcccacccctgggaggccggtagaggagcccctgctgactgcccgctctctggcctggcagcgtggagcagtgcaccttcatggactccaagatgaagcccctgtggatcatgtacagcaacgaggaggcaggcagcggcggcagcgtgggcatcatctttaagaacggggatggtgagggcctggcctccccacaccccgcctgtactgccctggggggtcctggggtgctcctagagtgggggtggagaagacagaatcctgggacttaagggcttgggtgtagctggaagcagagaacctaccagaaactcacgcttctcctcccaccggccggtggcacagacctccggcaggacatgctgaccctgcagatgatccagctcatggacgtcctgtg

SEQ ID NO: 26 - DNA, 18 bp, artificial
  PIK3CDExon8 F primer
ctgtgggactgccgtggg

SEQ ID NO: 27 - DNA, 20 bp, artificial
  PIK3CDExon8 R primer
tacccctccaggatacagcc

SEQ ID NO: 28 - DNA, 22 bp, artificial
  PIK3CDExon8 probe NHEJ
ccaggagccccaccttcatccg

SEQ ID NO: 29 - DNA, 20 bp, artificial
  PIK3CDExon17 F primer
gctgagctctcagaagaccc

SEQ ID NO: 30 - DNA, 20 bp, artificial
  PIK3CDExon17 R primer
gctcaccagacttcagccag

SEQ ID NO: 31 - DNA, 20 bp, artificial
  PIK3CDExon17 probe NHEJ
taggtaggcctcctgccgca

SEQ ID NO: 32 - DNA, 20 bp, artificial
  RPP30 F primer
agtctgtcgatggtgtgcag

SEQ ID NO: 33 - DNA, 21 bp, artificial
  RPP30 R primer
ggaggacatttgaggagtggt

SEQ ID NO: 34 - DNA, 24 bp, artificial
  RPP30 probe reference
cagtggtgtgagggagttatcact

SEQ ID NO: 35 - DNA, 23 bp, artificial
  PIK3CDExon24 F primer
ccgagtgaagtttaacaaagccc

SEQ ID NO: 36 - DNA, 20 bp, artificial
  PIK3CDExon24 R primer
aggtgcagttcaggctcttc

SEQ ID NO: 37 - DNA, 33 bp, artificial
  PIK3CDExon24 probe NHEJ5'
tttgttaaacttcactcggaagtgcttcagtgc

SEQ ID NO: 38 - DNA, 24 bp, artificial
  PIK3CDExon24 probe NHEJ3'
acaaagccctccgtgagagctgga

SEQ ID NO: 39 - DNA, 23 bp, artificial
  PIK3CDExon24 Reference probe
tgtttgcaggactccctggcact

SEQ ID NO: 40 - protein, 925 aa, artificial
  TALEN Exon8 Left
MGDPKKKRKVIDIADLRTLGYSQQQQEKIKPKVRSTVAQHHEALVGHGFTHAHIVALSQHPAALGTVAVKYQDMIAALPEATHEAIVGVGKQWSGARALEALLTVAGELRGPPLQLDTGQLLKIAKRGGVTAVEAVHAWRNALTGAPLNLTPQQVVAIASNNGGKQALETVQRLLPVLCQAHGLTPEQVVAIASNIGGKQALETVQALLPVLCQAHGLTPEQVVAIASNIGGKQALETVQALLPVLCQAHGLTPEQVVAIASHDGGKQALETVQRLLPVLCQAHGLTPQQVVAIASNNGGKQALETVQRLLPVLCQAHGLTPEQVVAIASHDGGKQALETVQRLLPVLCQAHGLTPEQVVAIASHDGGKQALETVQRLLPVLCQAHGLTPQQVVAIASNNGGKQALETVQRLLPVLCQAHGLTPEQVVAIASNIGGKQALETVQALLPVLCQAHGLTPEQVVAIASHDGGKQALETVQRLLPVLCQAHGLTPQQVVAIASNNGGKQALETVQRLLPVLCQAHGLTPEQVVAIASNIGGKQALETVQALLPVLCQAHGLTPQQVVAIASNNGGKQALETVQRLLPVLCQAHGLTPEQVVAIASHDGGKQALETVQRLLPVLCQAHGLTPQQVVAIASNNGGKQALETVQRLLPVLCQAHGLTPQQVVAIASNGGGRPALESIVAQLSRPDPALAALTNDHLVALACLGGRPALDAVKKGLGDPISRSQLVKSELEEKKSELRHKLKYVPHEYIELIEIARNSTQDRILEMKVMEFFMKVYGYRGKHLGGSRKPDGAIYTVGSPIDYGVIVDTKAYSGGYNLPIGQADEMQRYVEENQTRNKHINPNEWWKVYPSSVTEFKFLFVSGHFKGNYKAQLTRLNHITNCNGAVLSVEELLIGGEMIKAGTLTLEEVRRKFNNGEINFAAD

SEQ ID NO: 41 - protein, 925 aa, artificial
  TALEN Exon8 Right
MGDPKKKRKVIDIADLRTLGYSQQQQEKIKPKVRSTVAQHHEALVGHGFTHAHIVALSQHPAALGTVAVKYQDMIAALPEATHEAIVGVGKQWSGARALEALLTVAGELRGPPLQLDTGQLLKIAKRGGVTAVEAVHAWRNALTGAPLNLTPEQVVAIASHDGGKQALETVQRLLPVLCQAHGLTPEQVVAIASHDGGKQALETVQRLLPVLCQAHGLTPEQVVAIASHDGGKQALETVQRLLPVLCQAHGLTPEQVVAIASNIGGKQALETVQALLPVLCQAHGLTPEQVVAIASHDGGKQALETVQRLLPVLCQAHGLTPEQVVAIASHDGGKQALETVQRLLPVLCQAHGLTPQQVVAIASNGGGKQALETVQRLLPVLCQAHGLTPEQVVAIASNIGGKQALETVQALLPVLCQAHGLTPQQVVAIASNGGGKQALETVQRLLPVLCQAHGLTPEQVVAIASHDGGKQALETVQRLLPVLCQAHGLTPEQVVAIASHDGGKQALETVQRLLPVLCQAHGLTPEQVVAIASHDGGKQALETVQRLLPVLCQAHGLTPEQVVAIASNIGGKQALETVQALLPVLCQAHGLTPQQVVAIASNNGGKQALETVQRLLPVLCQAHGLTPQQVVAIASNNGGKQALETVQRLLPVLCQAHGLTPQQVVAIASNGGGRPALESIVAQLSRPDPALAALTNDHLVALACLGGRPALDAVKKGLGDPISRSQLVKSELEEKKSELRHKLKYVPHEYIELIEIARNSTQDRILEMKVMEFFMKVYGYRGKHLGGSRKPDGAIYTVGSPIDYGVIVDTKAYSGGYNLPIGQADEMQRYVEENQTRNKHINPNEWWKVYPSSVTEFKFLFVSGHFKGNYKAQLTRLNHITNCNGAVLSVEELLIGGEMIKAGTLTLEEVRRKFNNGEINFAAD

SEQ ID NO: 42 - protein, 925 aa, artificial
  TALEN Exon17 Left
MGDPKKKRKVIDIADLRTLGYSQQQQEKIKPKVRSTVAQHHEALVGHGFTHAHIVALSQHPAALGTVAVKYQDMIAALPEATHEAIVGVGKQWSGARALEALLTVAGELRGPPLQLDTGQLLKIAKRGGVTAVEAVHAWRNALTGAPLNLTPQQVVAIASNNGGKQALETVQRLLPVLCQAHGLTPEQVVAIASNIGGKQALETVQALLPVLCQAHGLTPQQVVAIASNGGGKQALETVQRLLPVLCQAHGLTPQQVVAIASNNGGKQALETVQRLLPVLCQAHGLTPEQVVAIASHDGGKQALETVQRLLPVLCQAHGLTPEQVVAIASNIGGKQALETVQALLPVLCQAHGLTPEQVVAIASHDGGKQALETVQRLLPVLCQAHGLTPQQVVAIASNGGGKQALETVQRLLPVLCQAHGLTPQQVVAIASNGGGKQALETVQRLLPVLCQAHGLTPQQVVAIASNNGGKQALETVQRLLPVLCQAHGLTPQQVVAIASNGGGKQALETVQRLLPVLCQAHGLTPQQVVAIASNNGGKQALETVQRLLPVLCQAHGLTPEQVVAIASHDGGKQALETVQRLLPVLCQAHGLTPEQVVAIASNIGGKQALETVQALLPVLCQAHGLTPQQVVAIASNGGGKQALETVQRLLPVLCQAHGLTPQQVVAIASNGGGRPALESIVAQLSRPDPALAALTNDHLVALACLGGRPALDAVKKGLGDPISRSQLVKSELEEKKSELRHKLKYVPHEYIELIEIARNSTQDRILEMKVMEFFMKVYGYRGKHLGGSRKPDGAIYTVGSPIDYGVIVDTKAYSGGYNLPIGQADEMQRYVEENQTRNKHINPNEWWKVYPSSVTEFKFLFVSGHFKGNYKAQLTRLNHITNCNGAVLSVEELLIGGEMIKAGTLTLEEVRRKFNNGEINFAAD

SEQ ID NO: 43 - protein, 925 aa, artificial
  TALEN Exon17 Right
MGDPKKKRKVIDIADLRTLGYSQQQQEKIKPKVRSTVAQHHEALVGHGFTHAHIVALSQHPAALGTVAVKYQDMIAALPEATHEAIVGVGKQWSGARALEALLTVAGELRGPPLQLDTGQLLKIAKRGGVTAVEAVHAWRNALTGAPLNLTPQQVVAIASNNGGKQALETVQRLLPVLCQAHGLTPQQVVAIASNNGGKQALETVQRLLPVLCQAHGLTPQQVVAIASNNGGKQALETVQRLLPVLCQAHGLTPEQVVAIASNIGGKQALETVQALLPVLCQAHGLTPQQVVAIASNNGGKQALETVQRLLPVLCQAHGLTPEQVVAIASNIGGKQALETVQALLPVLCQAHGLTPQQVVAIASNNGGKQALETVQRLLPVLCQAHGLTPQQVVAIASNNGGKQALETVQRLLPVLCQAHGLTPQQVVAIASNNGGKQALETVQRLLPVLCQAHGLTPEQVVAIASHDGGKQALETVQRLLPVLCQAHGLTPEQVVAIASHDGGKQALETVQRLLPVLCQAHGLTPQQVVAIASNGGGKQALETVQRLLPVLCQAHGLTPEQVVAIASHDGGKQALETVQRLLPVLCQAHGLTPQQVVAIASNGGGKQALETVQRLLPVLCQAHGLTPEQVVAIASNIGGKQALETVQALLPVLCQAHGLTPQQVVAIASNGGGRPALESIVAQLSRPDPALAALTNDHLVALACLGGRPALDAVKKGLGDPISRSQLVKSELEEKKSELRHKLKYVPHEYIELIEIARNSTQDRILEMKVMEFFMKVYGYRGKHLGGSRKPDGAIYTVGSPIDYGVIVDTKAYSGGYNLPIGQADEMQRYVEENQTRNKHINPNEWWKVYPSSVTEFKFLFVSGHFKGNYKAQLTRLNHITNCNGAVLSVEELLIGGEMIKAGTLTLEEVRRKFNNGEINFAAD

SEQ ID NO: 44 - protein, 925 aa, artificial
  TALEN Exon24 Left
MGDPKKKRKVIDIADLRTLGYSQQQQEKIKPKVRSTVAQHHEALVGHGFTHAHIVALSQHPAALGTVAVKYQDMIAALPEATHEAIVGVGKQWSGARALEALLTVAGELRGPPLQLDTGQLLKIAKRGGVTAVEAVHAWRNALTGAPLNLTPQQVVAIASNNGGKQALETVQRLLPVLCQAHGLTPQQVVAIASNNGGKQALETVQRLLPVLCQAHGLTPEQVVAIASHDGGKQALETVQRLLPVLCQAHGLTPEQVVAIASNIGGKQALETVQALLPVLCQAHGLTPEQVVAIASHDGGKQALETVQRLLPVLCQAHGLTPQQVVAIASNGGGKQALETVQRLLPVLCQAHGLTPQQVVAIASNNGGKQALETVQRLLPVLCQAHGLTPQQVVAIASNNGGKQALETVQRLLPVLCQAHGLTPQQVVAIASNNGGKQALETVQRLLPVLCQAHGLTPQQVVAIASNNGGKQALETVQRLLPVLCQAHGLTPEQVVAIASNIGGKQALETVQALLPVLCQAHGLTPEQVVAIASNIGGKQALETVQALLPVLCQAHGLTPEQVVAIASNIGGKQALETVQALLPVLCQAHGLTPEQVVAIASNIGGKQALETVQALLPVLCQAHGLTPEQVVAIASHDGGKQALETVQRLLPVLCQAHGLTPQQVVAIASNGGGRPALESIVAQLSRPDPALAALTNDHLVALACLGGRPALDAVKKGLGDPISRSQLVKSELEEKKSELRHKLKYVPHEYIELIEIARNSTQDRILEMKVMEFFMKVYGYRGKHLGGSRKPDGAIYTVGSPIDYGVIVDTKAYSGGYNLPIGQADEMQRYVEENQTRNKHINPNEWWKVYPSSVTEFKFLFVSGHFKGNYKAQLTRLNHITNCNGAVLSVEELLIGGEMIKAGTLTLEEVRRKFNNGEINFAAD

SEQ ID NO: 45 - protein, 925 aa, artificial
  TALEN Exon24 Right
MGDPKKKRKVIDIADLRTLGYSQQQQEKIKPKVRSTVAQHHEALVGHGFTHAHIVALSQHPAALGTVAVKYQDMIAALPEATHEAIVGVGKQWSGARALEALLTVAGELRGPPLQLDTGQLLKIAKRGGVTAVEAVHAWRNALTGAPLNLTPQQVVAIASNNGGKQALETVQRLLPVLCQAHGLTPQQVVAIASNGGGKQALETVQRLLPVLCQAHGLTPQQVVAIASNGGGKQALETVQRLLPVLCQAHGLTPEQVVAIASNIGGKQALETVQALLPVLCQAHGLTPEQVVAIASNIGGKQALETVQALLPVLCQAHGLTPEQVVAIASNIGGKQALETVQALLPVLCQAHGLTPEQVVAIASHDGGKQALETVQRLLPVLCQAHGLTPQQVVAIASNGGGKQALETVQRLLPVLCQAHGLTPQQVVAIASNGGGKQALETVQRLLPVLCQAHGLTPEQVVAIASHDGGKQALETVQRLLPVLCQAHGLTPEQVVAIASNIGGKQALETVQALLPVLCQAHGLTPEQVVAIASHDGGKQALETVQRLLPVLCQAHGLTPQQVVAIASNGGGKQALETVQRLLPVLCQAHGLTPEQVVAIASHDGGKQALETVQRLLPVLCQAHGLTPQQVVAIASNNGGKQALETVQRLLPVLCQAHGLTPQQVVAIASNGGGRPALESIVAQLSRPDPALAALTNDHLVALACLGGRPALDAVKKGLGDPISRSQLVKSELEEKKSELRHKLKYVPHEYIELIEIARNSTQDRILEMKVMEFFMKVYGYRGKHLGGSRKPDGAIYTVGSPIDYGVIVDTKAYSGGYNLPIGQADEMQRYVEENQTRNKHINPNEWWKVYPSSVTEFKFLFVSGHFKGNYKAQLTRLNHITNCNGAVLSVEELLIGGEMIKAGTLTLEEVRRKFNNGEINFAAD

SEQ ID NO: 46 - protein, 1044 aa, homosapiens
  PI3Kdelta isoform 1
MPPGVDCPMEFWTKEENQSVVVDFLLPTGVYLNFPVSRNANLSTIKQLLWHRAQYEPLFHMLSGPEAYVFTCINQTAEQQELEDEQRRLCDVQPFLPVLRLVAREGDRVKKLINSQISLLIGKGLHEFDSLCDPEVNDFRAKMCQFCEEAAARRQQLGWEAWLQYSFPLQLEPSAQTWGPGTLRLPNRALLVNVKFEGSEESFTFQVSTKDVPLALMACALRKKATVFRQPLVEQPEDYTLQVNGRHEYLYGSYPLCQFQYICSCLHSGLTPHLTMVHSSSILAMRDEQSNPAPQVQKPRAKPPPIPAKKPSSVSLWSLEQPFRIELIQGSKVNADERMKLVVQAGLFHGNEMLCKTVSSSEVSVCSEPVWKQRLEFDINICDLPRMARLCFALYAVIEKAKKARSTKKKSKKADCPIAWANLMLFDYKDQLKTGERCLYMWPSVPDEKGELLNPTGTVRSNPNTDSAAALLICLPEVAPHPVYYPALEKILELGRHSECVHVTEEEQLQLREILERRGSGELYEHEKDLVWKLRHEVQEHFPEALARLLLVTKWNKHEDVAQMLYLLCSWPELPVLSALELLDFSFPDCHVGSFAIKSLRKLTDDELFQYLLQLVQVLKYESYLDCELTKFLLDRALANRKIGHFLFWHLRSEMHVPSVALRFGLILEAYCRGSTHHMKVLMKQGEALSKLKALNDFVKLSSQKTPKPQTKELMHLCMRQEAYLEALSHLQSPLDPSTLLAEVCVEQCTFMDSKMKPLWIMYSNEEAGSGGSVGIIFKNGDDLRQDMLTLQMIQLMDVLWKQEGLDLRMTPYGCLPTGDRTGLIEVVLRSDTIANIQLNKSNMAATAAFNKDALLNWLKSKNPGEALDRAIEEFTLSCAGYCVATYVLGIGDRHSDNIMIRESGQLFHIDFGHFLGNFKTKFGINRERVPFILTYDFVHVIQQGKTNNSEKFERFRGYCERAYTILRRHGLLFLHLFALMRAAGLPELSCSKDIQYLKDSLALGKTEEEALKHFRVKFNEALRESWKTKVNWLAHNVSKDNRQ